European Patent Specification EP 3 589 645 B1, published August 2, 2023. Title: Cyclic peptides for the treatment of Graves  disease. Applicant: advanceCor GmbH. The sequence listing filed with the application follows.

SEQUENCE LISTING (10 sequences)

SEQ ID NO: 1 - protein, 24 aa, artificial
  Amino acid sequence derived from human thyrotropin-TSH receptor (TSHR)
GYAFNGTKLDAVYLNKNKYLTVID

SEQ ID NO: 2 - protein, 24 aa, artificial
  Amino acid sequence derived from human thyrotropin-TSH receptor (TSHR)
SPPCECHQEEDFRVTCKDIQRIPS

SEQ ID NO: 3 - protein, 24 aa, artificial
  Amino acid sequence derived from human thyrotropin-TSH receptor (TSHR)
LPPSTQTLKLIETHLRTIPSHAFS

SEQ ID NO: 4 - protein, 17 aa, artificial
  Amin acid sequence derived from human thyrotropin-TSH receptor (TSHR)
SNLPNISRIYVSIDVTL

SEQ ID NO: 5 - protein, 24 aa, artificial
  Amin acid sequence derived from human thyrotropin-TSH receptor (TSHR)
YNLSKVTHIEIRNTRNLTYIDPDA

SEQ ID NO: 6 - protein, 24 aa, artificial
  Amin acid sequence derived from human thyrotropin-TSH receptor (TSHR)
LKELPLLKFLGIFNTGLKMFPDLT

SEQ ID NO: 7 - protein, 17 aa, artificial
  Amin acid sequence derived from human thyrotropin-TSH receptor (TSHR)
KVYSTDIFFILEITDNP

SEQ ID NO: 8 - protein, 24 aa, artificial
  Amin acid sequence derived from human thyrotropin-TSH receptor (TSHR)
NAFQGLCNETLTLKLYNNGFTSVQ

SEQ ID NO: 9 - protein, 20 aa, artificial
  Amin acid sequence derived from human thyrotropin-TSH receptor (TSHR)
KDAFGGVYSGPSLLDVSQTS

SEQ ID NO: 10 - protein, 24 aa, artificial
  Amin acid sequence derived from human thyrotropin-TSH receptor (TSHR)
PSKGLEHLKELIARNTWTLKKLPL